European Patent Specification EP 4 104 853 B1, published May 6, 2026. Title: ARGININE DEIMINASE WITH REDUCED CROSS-REACTIVITY TOWARD ADI - PEG 20 ANTIBODIES FOR CANCER TREATMENT. Applicant: Polaris Group. The sequence listing filed with the application follows.

SEQUENCE LISTING (28 sequences)

SEQ ID NO: 1 - protein, 409 aa, Mycoplasma hominis
MSVFDSKFNGIHVYSEIGELETVLVHEPGREIDYITPARLDELLFSAILESHDARKEHQSFVKIMKDRGINVVELTDLVAETYDLASKAAKEEFIETFLEETVPVLTEANKKAVRAFLLSKPTHEMVEFMMSGITKYELGVESENELIVDPMPNLYFTRDPFASVGNGVTIHFMRYIVRRRETLFARFVFRNHPKLVKTPWYYDPAMKMPIEGGDVFIYNNETLVVGVSERTDLDTITLLAKNIKANKEVEFKRIVAINVPKWTNLMHLDTWLTMLDKNKFLYSPIANDVFKFWDYDLVNGGAEPQPQLNGLPLDKLLASIINKEPVLIPIGGAGATEMEIARETNFDGTNYLAIKPGLVIGYDRNEKTNAALKAAGITVLPFHGNQLSLGMGNARCMSMPLSRKDVKW

SEQ ID NO: 2 - protein, 410 aa, Mycoplasma salivarium
MSVFSSKFNGIHVYSEIGELETVLVHEPGKEIDYITPSRLDELLFSAILESHDARKEHQEFVATLKKEKINVVELTDLVTETYDLVDQKTKDKLIDEFLEDSEPVLTAELKATVKKFLKSFKETRKLIEVMMAGITKYDLGIKADRELIVDPMPNLYFTRDPFASVGNGVTIHYMRYKVRQRETLFSRFIFNNHPKLVKTPWYYDPAMKMSIEGGDVFIYNNDTLVVGVSERTDLDTITLLAKNIKANKECEFKRIVAINVPKWTNLMHLDTWLTMLDKDKFLYSPIANDIFKFWDYDLVNGGANPQPKDNGLPLDKLLKSIIGKEPVLIPIAGHHATEIEVARETHFDGTNYLAIRPGVVIGYARNEKTNEALKDAGITVLPFKGNQLSLGMGNARCMSMPLSRKDVKW

SEQ ID NO: 3 - protein, 411 aa, Mycoplasma spumans
MSVFDSKFKGIHVYSEIGELESVLVHEPGREIDYITPARLDELLFSAILESHDARKEHKGFVAELKKQNVNVIELTDLVAETYELASKEAQAKLIEDFIEDSEPVLNAEEAQAVRKFLSERKSTREMVEYMMSGLTKYELGLESADRELIVDPMPNLYFTRDPFASVGNGVTIHYMKYKVRQRETLFAKFVFSNHPKLVNTPRYYDPSMKLPIEGGDVFIYNNETLVVGCSERTELETITLLAKNIKANKEVEFKRIVAINVPKWTNLMHLDTWLTMLDKDKFLYSPIANDVFKFWDYDLVNGGEEPQPVENGLPLEELLASIINKKPTLIPIAGEGATHIDVERETHFDGTNYLAIAPALIIGYSRNEKTNAALEKAGITVLPFHGNQLSLGMGNARCMSMPLSRKDVKW

SEQ ID NO: 4 - protein, 410 aa, Mycoplasma auris
MSVFDSKFKGIHVYSEIGELETVLVHEPGREIDYITPKRLDELLFSAILESHEARKEHKQFVAELKANDINVVELTDLVAETYDLVSQELKDKLIEEFLDDSYPVLTEEHKKAVRSFLKSRSSTRELIEYMMAGITKYDLGIEAEGDLIVDPMPNLYFTRDPFASVGNGVTIHYMRYKVRQRETLFSRFIFDNHPKLVNTPRYYDPSLKLSIEGGDVFIYNNDTLVMGVSERTDLETVTLLAKNIVANKECEFKRIVAINVPHWTNLMHLDTWLTMLDKDKFLYSPIANDYFKFWDYDLVNGGAEPQPVVNELPLDKLLESIIHKKPILIPIAGEGASQIDLERETHFDGTNYLVLRPGVVVGYARNEKTNAALEAVGIKVLPFYGNQLSLGMGNSRCMSMPLSRKDVKW

SEQ ID NO: 5 - protein, 410 aa, Mycoplasma hyosynoviae
MSVFNSKFKGIHVYSEIGDLESVLVHEPGKEIDYITPSRLDELLFSAILESNDARKEHKEFVEILKKEGVNVVELVDLIAETIDLVDAKKKEALIDEYIEDSEPVVDAKVKPLVKKLLLGIKDTKELVKLMMAGITKYDLEIESEKELIIDPMPNLYFTRDPFASVGNGVTIHYMRYKVRQRETLFSRFVFRNHPKLTSTPWYYDPAMKLSIEGGDVFIYNNDTLVVGVSERTDLDTITLLAKNIKANKECEFKRIVAINVPKWTNLMHLDTWLTMLDKDKFLYSPIANDIFKFWDYDLVNGGSEPQPKDNGLPLEKLLESIIGKKPVLIPIAGCCASDIEIARETHFDGTNYLAIKPGVVIGYARNEKTNKALEKAGIKVLPFKGNQLSLGMGNARCMSMPLSRKDVKW

SEQ ID NO: 6 - protein, 409 aa, Mycoplasma cloacale
MSVFDKRFKGIHVYSEIGELQTVLVHEPGREIDYITPARLDELLFSAILESHDARKEHKEFVKILESQGINVVELTDLIAETYELASEEAKDNLIEEFLDESEPVLSEEHRILVRNFLKGITKTKELVKMMMAGITKYDLGIEADRELIVDPMPNLYFTRDPFASVGNGVTIHYMRYKVRQRETLFSRFIFENHPKLVSTPIYYHPSQGLSIEGGDVFIYNNDTLVVGVSERTDLQTITLLAKNIKANEECEFKRIVAINVPKWTNLMHLDTWLTMLDKNKFLYSPIANDVFKFWDYDLVNGGDEPQPVDNGLPLNELLASIIGEEPVLVPIAGEGASKMDIERETHFDGTNYLAIAPGVVVGYSRNEKTNAALEKAGIKVLPFKGHQLSLGMGNARCMSMPLYRKDVK

SEQ ID NO: 7 - protein, 412 aa, Mycoplasma alkalescens
MSVFDSKFKGIHVYSEIGELESVLVHEPGHEIDYITPSRLDELLFSAMLESHDARKEHKQFVAELKANNVNVIELTDLVAETYDLASQEAKDKLIEEFLEDSEPVLSEENKIAVRDFLKSRKTTRELIEVMMAGITKYDLGIKNCKCQDLVVDPMPNLYFTRDPFASVGNGITIHYMRYKVRQRETLFSRFIFANHPKLVNTPIYYHPSLKLSIEGGDVFIYNNDTLVVGVSERTDLETITLLAKNIVANKECEFKRIVAINVPKWTNLMHLDTWLTMLDKDKFLYSPIANDVFKFWDYDLVNGGAEPKPVENGSSLEAILESIIHKKPILIPIGGDSASQIEVERETHFDGTNYLAIRPGVVIGYSRNVKTNAALEAAGIKVIPFHGNQLSLGMGNARCMSMPLSRKDVKW

SEQ ID NO: 8 - protein, 410 aa, Mycoplasma orale
MSVFSDKFNGIHVYSEIGDLESVLVHEPGKEIDYITPARLDELLFSAILESTDARKEHKEFVEILKKQGINVVELVDLVVETYNLVDKKTQEKLLKDFLDDSEPVLSPEHRKAVEKFLKSLKSTKELIQYMMAGITKYDLGIKADKELIVDPMPNLYFTRDPFASVGNGVTIHYMRYKVRQRETLFSKFIFTNHPKLVKTPWYYDPAMKLSIEGGDVFIYNNDTLVVGVSERTDLETITLLAKNIKANKECEFKRIVAINVPKWTNLMHLDTWLTMLDKDKFLYSPIANDVFKFWDYDLVNGGSNPEPVVNGLPLDKLLESIINKKPVLIPIAGKGATEIETAVETHFDGTNYLAIKPGVVVGYSRNVKTNAALEANGIKVLPFKGNQLSLGMGNARCMSMPLSRKDVKW

SEQ ID NO: 9 - protein, 401 aa, Mycoplasma iners
MSKINVYSEIGVLKEVLVHTPGDEIRRIAPSRLDELLFSAILEPSAAIQEHKSFLKILQDRGIKTIQLSDLVAETYKHYASEAEKEAFIEKYLDEATPVLSKDMRAKVKNYILSMQGEPVKMVRTMMAGVSKQELNVESEVELIVDPMPNLYFTRDPFASAGNGISLNNMKYVVRKRETIFAEFIFSIHPEYKKTPHWFDRLDNGSIEGGDVFIYNKDTLVIGVSERTNKEAIITIAKHIQDNKEAQFKKIVAINVPPMPNLMHLDTWLTMVDKNKFLYSPNMLSVLKVWEIDLSKPIEMVETNKPLAEVLESIIGEKPILIPIAGKDATQLDIDIETHFDGTNYLTIAPGVVVGYSRNVKTEAALRAAGVTVLSFEGNQLSLGMGSARCMSMPLVREDVK

SEQ ID NO: 10 - protein, 401 aa, Mycoplasma gallinarum
MSKIRVYSEIGNLKKVLVHTPGDEIRRISPSRLEELLFSAVLEPNAAIEEHKRFVKLLEDRGIQAIQLSDLVAETYVKYATAEQKAAFIEKYLDEATPALSAENRERAKKYILSLEMQPVKMIRTMMAGLSKYELNVESNIELIIDPMPNLYFTRDPFASAGNGISLNNMKYVVRKRETIFAEFIFAIHPEYKETPHWFDRLDHGSIEGGDVFVYNKDTLVIGVSERTNKEAIITIAKHIQDNKEAEFKKIVAINVPPMPNLMHLDTWLTMVDKNKFIYSPNMLSVLKIWEIDLAKPIEMVESNKSLTEVLESIIGEKPILIPIAGEGASQLDIDIETHFDGTNYLTIAPGVVVGYSRNEKTEKALKAAGITVLSFEGNQLSLGMGSARCMSMPLVREDVK

SEQ ID NO: 11 - protein, 405 aa, Mycoplasma pirum
MNSNQKGIHVYSEIGKLKEVLVHRPGRELDFLDPTRLDELLFAATLEAETARLEHDNFTNALKNQGVTVIELADLVAQTYSSSTPTIKAAFINKYLDEATPALTTKLRTLVKDFLTKQKSVRKMVDYMIGGILSTDLNIKGKPELIVEPMPNAYFTHDPFASVGNGVTLHYMKHNVRRREVLFSEFIFNNNERFQNTPRYIVPTKGLDIEGGDVFVYNKNTLVVGVSERTKMVTIKELAKNILKNKECLFKKIYAINVPKMPNLMHLDTWLTMLDHNKFLYSPNMLSVLKIWEIDISSGKSISSPKELNMDLSKALSIIIGKKPILIPVAGENASQIDINIETNFDATNYLVTQPGVVVGYSRNKKTEAALIKAGIEVIPFQGNQLSLGMGSARCMSMPLIREDV

SEQ ID NO: 12 - protein, 404 aa, Mycoplasma primatum
MSKSKINVYSEYGNLKEVLVHTPGDEIRRITPSRLDELLFSAILEPKSAIAEHKSFCQILKDNKVKAIQLDELVAATYKGVSESVQNSFVERWLDECEPKLENNVRPIVKEYLLKAAEQSVKKMIRIMMAGIDKREIGVESEVDFIVDPMPNLYFTRDPFASVGNGITLHHMKYVVRQRETLFSEFIFDNHPDYKFVPRYFDRDDEGKIEGGDVFIYNSKTLVVGISERTNKDAIRIVAKKIQANADAKFEKIFAINVPPMPNLMHLDTWLTMLDSNKFLYSPNMLSVLKVWEINLDDPALEWKEISGSLEEILTYIIGKKPILIPIAGKGASQFEIDIETHFDGTNYLAIAPSVVIGYSRNELTEKALKKAGVKVLSLDGNQLSLGMGSARCMSMPLIREDVK

SEQ ID NO: 13 - protein, 401 aa, Mycoplasma lipofaciens
MSKINVYSEVGVLKEVLVHTPGDEIRRVAPSRLDELLFSAILEPQDAIAEHKRFIKILEDNNIKVIQLDELVSETWEKATAEQRDAFIEKWLDEAEPVLDAKLRETVKKYLLSLNPVKKMVRTMMAGIDKKELKIELDRDLVVDPMPNLYFTRDPFASAGNGISLNNMKYVTRKRETIFAEFIFNIHPDYKTTPHWFDRLDKGNIEGGDVFIYNKDTLVLGVSERTNKDAVMTIAKHIQSNEQAKFKKLVAINVPPMPNLMHLDTWLTMVDHDKFLYSPNMLSVLKIWEIDLTPGKEIEMVESTKSLSDMLESIIGKKPVLIPIAGKDASQLDIDIETHFDGTNYLTIRPGVVVGYSRNCLTEQALKDAGVTVLSFDGNQLSLGMGSARCMSMPLVREDIK

SEQ ID NO: 14 - protein, 405 aa, Mycoplasma felifaucium
MNKINVYSEIGKLKEVLVHTPGNEIRRISPSRLDELLFSALLEPNFAAKEHTAFCEILKENGIKAIQLVDLVSDTWRIASEKAKTEFIERWLDECEPKLDSNLREIVRKHIYAIEKRSVKRMVKTMMAGIERRELPVTSKEVARELVVDPMPNLYFTRDPFASVGNGISLHHMKYVTRQRETIFAEFVFGNHPDYIDTPRWFDRSDDGRIEGGDVFIYGSKTLVIGVSERTNKEAIKVMAKKIQANKEATFEKIYAINVPPMPNLMHLDTWLTMLDKNKFLYSPNMLAVLQVWEIDLKDPELTWHELSGSLEEILHKIIGRKPILIPIAGHGAQQIDIDIETHFDGTNYLAIAPGVVVGYNRNVLTERALKKAGIKVLSFEGNQLSLGMGSARCMSMPLIRENLK

SEQ ID NO: 15 - protein, 404 aa, Mycoplasma imitans
MFNKIKVYSEIGRLRKVLVHTPGKELEYVTPQRLDELLFSSLLNPVKARQEHEAFIKILQDQGVECVQLTTLTAQTFQSATSEVKEKFINRWLDECLPKLSDDNRIKVYAYLKDLSSDPEVMIRKMMSGILAKEVNVQSDVELIADPMPNLYFTRDPFASIGKGVTLHSMFHPTRKRETIFADFVFSHHPEYKQTPKYYSRLNEYSIEGGDLFVYDDKTLVIGVSERTEKKAIQFLAEKLRENYETTFEKIYAINVPKMSNLMHLDTWLTMLDYDKFLYSPNMMGVLKIWEIDLTHEQLSWRELNESLEEFLSMVIGKKATTIPVAGEDSTQIEIDVETNFDATNFLVIQPGVVVGYDRNYKTNQALVNAGIKVLSWNGDQLSLGMGSARCMSMPLYRDPIKKG

SEQ ID NO: 16 - protein, 401 aa, Mycoplasma opalescens
MSKINVYSEIGTLKEVLVHTPGDEIRRVAPARLDELLFSAILEPNHAIAEHKAFIKILEDNGIKVIQLDELVVQTWNQVDEATRKAFVTKWLDECEPKLESNVRVEVEKYIYSLAKEPKKMVRTMMAGISKEELPLNVNRPLVVDPMPNLYFTRDPFASVGTGISLHHMKYVTRQRETIFAQFVFDNHKDYNTVPRWFDNKDQGRIEGGDVFIYNTKTLVIGVSERTDKDAIKIMAKKIQADKNCKFEKIFAINVPPMPNLMHLDTWLTMVDRNKFLYSPNMLSVLKVWEIDLKDASLAWKEIEGSLSQILEKIIGEKPILIPIAGENASQLDIDIETHFDGTNYLTIAPGVVVGYSRNVKTEQALKAAGVKVLSFEGNQLSLGMGSARCMSMPLIREDLK

SEQ ID NO: 17 - protein, 431 aa, Mycoplasma moatsii
MGIKKIMKKNAINVYSEIGKLKKVLVHRPGDELKYVTPQRMDELLMSAIIELEQAKEEHDAFTKILRDNGVEVIELADLTAEMYDSLTPSEKDAFLNQWVKEASWGKKSSIDALKIKKNLSKKVFDYVKSIKPTRKMIDKLMAGVLLSEIGEKSIILNKDKKNEMVIDLVVDPMPNLYFTRDPFASVGNGITLHNMKYPTRKRETIFAQWIFNKHPEYKDVPQFISKRDGKETIEGGDVFIYTKDVLAIGVSERTNMEAILRIATNIKKDKNCEFKKIVAINVPPMGNLMHLDTWLTMLDKDLFLYSGNIKSALKVWEIDLTKPITPKSPKLSTAKLADILAKIVGKKVRMIPIGGKDGNQMDIDIETHFDGTNYLAIAPGVVVGYHRNRKTQKALEEAGVKVLAFQGNQLSLGMGSARCMSMPLVREEVK

SEQ ID NO: 18 - protein, 399 aa, Mycoplasma elephantis
MSQINVFSEIGQLKEVLVHTPGDEIRRISPKRYNELLFSAILEADVAIKEHKSFVKILEENNVKVIQLKDILLETWNICSKEAKNIFINKWIEEAQPVIHSSSLKEKIKLFLKSKTPLEIIDIMMKGILKQELGIEYKHELIIDPMPNLYFTRDPFTSMGSGITINNMKYQTRKRETIFSEFIFNNHPKYKNTPRWFDRFDSGNIEGGDLFVYTKETIVVGVSERTKKKAILKIAKNIQENNNSFKKIVVIKVPIMQNLMHLDTWIVMVDFDKFIYSPNVTKSLKFWEIDLTKKPKFIQLKNETLEDVLYRVIGKKPILIPVAGENANQIDIDVETHFDATNYLTIRPGVVVGYSRNKKTEEALINAGVKVYAFEGNQLSLGMGSARCMSMPLIREDII

SEQ ID NO: 19 - protein, 399 aa, Mycoplasma testudinis
MKNINVYSEVGKLKEVVVHTPGEELHNVAPSRLQELLTSAVLEPEVARKEHLKFIKILNDYGVKVIQIVDLITETYEAVDSNKKEAFINNWLDNSVPKLTDKNRMILRNYLTQFSTKAMIRKMISGIRAKELNLKTPSALLVDPMPNLCFARDTFACVGSAISLSTMKHPTRRREALLTEFIFQNHPKYKDVIKYFDSKNSKATIEGGDIFVYNPKTLVVGNSERTNMQACLLLAKKIQSNPNNKFEKIVIVNVPPLPHLMHLDTWLTMVDYDKFIYSPNILHTLKFWVIDLKKRKLEAVEKHNTLKAMLRMIIKKEPILIPVGDVGADQLDIDLETHFDATNYLALAPGVVVGYDRNIKTQRALEKAGVKVLSFSGNQLSLAMGSARCLSMPLIREEN

SEQ ID NO: 20 - protein, 410 aa, Mycoplasma canadense
MSVFDSKFKGIHVYSEIGELESVLVHEPGREIDYITPARLDELLFSAILESHDARKEHKQFVSELKANDINVVELTDLVAETYDLASQEAKDKLIEEFLEDSEPVLSEEHKAIVRKYLKGIQPTRKLIEMMMAGITKYDLGIEADHELIVDPMPNLYFTRDPFASVGNGVTIHYMRYKVRQRETLFSRFVFSNHPKLVNTPWYYDPSLKLSIEGGDVFVYNNDTLVVGVSERTDLQTVTLLAKNIVANKECEFKRIVAINVPKWTNLMHLDTWLTMLDKDKFLYSPIANDVFKFWDYDLVNGGSEPQPVENGLPLEGLLESIINKKPILIPIAGEGASQMEIERETHFDGTNYLAIRPGVVIGYSRNEKTNAALEAAGIKVLPFHGNQLSLGMGNARCMSMPLSRKDVKW

SEQ ID NO: 21 - protein, 409 aa, Mycoplasma anseris
MSVFDKRFKGIHVYSEIGELQTVLVHEPGREIDYITPARLDELLFSAILESHDARAEHKKFVATLKEQGINTVELTDLVAETYDLASQEARDNLLEEFLDDSAPVLSEEHKEIVRTYLKGIKGTRKLIETMMAGITKYDLGIEAEQELIVDPMPNLYFTRDPFASVGNGVTIHYMRYKVRQRETLFSRFIFSNHPQLVNTPWYYNPAEGLSIEGGDVFIYNNDTLVVGVSERTDLQTITLLAKNIKANEECEFKRIVAINVPKWTNLMHLDTWLTMLDTNKFLYSPIANDVFKFWDYDLVNGGDEPQPVDNGLPLNELLKSIIGEEPILIPIAGDGATQIEIERETHFDGTNYLAIAPGVVIGYSRNEKTNAALEAAGIKVLPFKGHQLSLGMGNARCMSMPLYRKDVK

SEQ ID NO: 22 - protein, 401 aa, Mycoplasma meleagridis
MSKINVYSEIGVLKEVLVHTPGDEIRRISPSRLDELLFSAILQPEQAIKEHQSFVKILQDRGIKVIQLSDLVAETYVKYATSKEKESFIEKWLDEATPALNSENRARVKNYITAMQGQPVKMVRAMMAGVSKQELNIESDVELIVDPMPNLYFTRDPFASAGNGISLNNMKYVVRKRETIFAEFIFSIHPEYKQTPHWFDRLDKGNIEGGDVFIYNKDTLVIGVSERTNKEAILTIAEHIKNNKEAKFKKIVAINVPPMPNLMHLDTWLTMVDKNKFLYSPNMLSVLKIWEIDLSKEIKMVETSKPLADVLESIIGEKPILIPIAGENASQLDIDIETHFDGTNYLTIAPGVVVGYSRNVKTEAALKAAGVTVYSFDGNQLSLGMGSGRCMSMPLVREDVK

SEQ ID NO: 23 - protein, 404 aa, Mycoplasma alvi
MSIKENGIHVYSEIGKLRDVLVHRPGRELNFLDPSRLDELLFAATLEPETARLEHDNFTTVLKNQGVNVIELADLVSQTYSKVDSKVKKEFIDQYLNEATPKLTSELSKKVYDFLTKQKSNREMVDFMMGGILSSDLNIKGQPYLIVEPMPNLYFTRDPFASVGNGATIHWMKHNVRRREVLFANFIFKYNERFQNTPKYITPTKGLDIEGGDVFVYNKKTLVVGVSERTKMETIKELAKNISKNKECTFTKIYAINVPKMPNLMHLDTWLTMLDYNKFLYSPNMLSVLKVWEINISNNKVSAPKELNVNLEKALSMIIGKKPILIPVAGANASQIDINIETNFDATNYLVIEPGVVVGYSRNKKTEEALVKAGIKVLPFHGNQLSLGMGSARCMSMPLYREDV

SEQ ID NO: 24 - protein, 410 aa, Mycoplasma penetrans
MSSIDKNSLGNGINVYSEIGELKEVLVHTPGDEIRYTAPSRLEELLFSAVLKADTAIEEHKGFVKILQNNGIKVIQLCDLVAETYELCSKEVRNSFIEQYLDEALPVLKKEIRPVVKDYLLSFPTVQMVRKMMSGILANELNIKQDNPLIIDGMPNLYFTRDPFASMGNGVSINCMKYPTRKREVIFSRFVFTNNPKYKNTPRYFDIVGNNGTIEGGDIFIYNSKTLVIGNSERTNFAAIESVAKNIQANKDCTFERIVVINVPPMPNLMHLDTWLTMLDYDKFLYSPNMMNVLKIWEIDLNVKPVKFVEKKGTLEEVLYSIIDKKPILIPIAGKGANQLDIDIETHFDGTNYLTIAPGVVVGYERNEKTQKALVEAGIKVLSFNGSQLSLGMGSARCMSMPLIRENLKK

SEQ ID NO: 25 - protein, 404 aa, Mycoplasma fermentans
MKKINVYSEYGKLKEVLVHTPGDEIRRIAPSRLDELLFSAILEPDSAIAEHKRFVQLLKDNGIKVIQLDELFAKTFDLVSESVKQSFIERWLDECEPKLDATLRAKVKEYILELKAKSSKKMVRVMMAGIDKKELGIELDRDLVVDPMPNLYFTRDPFASVGNGISLHHMKYVTRQRETIFSEFIFDNNLDYNTVPRWFDRKDEGRIEGGDVFIYSADTLVVGVSERTNKEAINVMARKIAADKEVKFKRIYAINVPPMPNLMHLDTWLTMLDKNKFLYSPNMLSVLKVWRIDLNDPDFVWHEIEGSLEEILEQIIGMKPILIPIAGKGASQLDIDIETHFDGTNYLTIAPSVVVGYSRNEKTEKALKAAKVKVLSFEGNQLSLGMGSARCMSMPLIREDIKKK

SEQ ID NO: 26 - protein, 404 aa, Mycoplasma pneumoniae
MKYNINVHSEIGQLQTVLVHTPGNEIRRISPRRLDDLLFSAVIEPDTAIQEHQTFCQLLQEQNIEVVQLTDLTATTFDKANATAQNQFIETWLDQAEPKLTPEHRKVAKQYLLEQKAKSTLSMVRSMMGGIDKRKVAAANTINGDFLVDPMPNLYFTRDPFASIGHGISINRMKYLTRRRETLFASFIFANHPIIAARKFYFKPIDMGTIEGGDIFVYDQQTVVMGLSERTTEAAINVLAKKIQQDSSTSFKRIFVINVPQLPNLMHLDTWLTMLDRNKFLYSPNMLAVLKAWRIDFTDPALKWNEIAGDLSTILHTIIGQKPMLIPIAGADANQTEIDIETHFDGTNYLTIAPSVVVGYARNKLTHQTLEAAGVKVIAFKGNQLSLGMGSARCMSMPLVRKPL

SEQ ID NO: 27 - protein, 414 aa, Mycoplasma sp.
MEKIHVTSEIGPLKKVLLHRPGNELLNLTPDTLSRLLFDDIPYLPDAIKEHDEFADALRANGVEVVYLENLMADVLDLSDEIRDKFIKQFIYEAGIRTPKYKYLVFDYLDQITNSKKLVLKTMEGIQISDIPRRKREIEKSLVDLIETEDEFIADPMPNLYFTRDPFASVGEGISLNKMYSVTRNRETIYAEYIFKYHPDYKDQARLYYDRYNPYHIEGGDVLNINDHVLAIGISQRTTAEAIDQIAKNLFKDPECKIDTILAFNIPESRAFMHLDTVFTQVDYDKFTYHPGIMGTLQVFEITEGDDPNSDEDLTVTEINAPLEEILTKYVGRKVTLIPCAGGDKVSAEREQWNDGSNTLCIAPGVVVVYDRNNLTNAVLRSYGLKVIEIHGAELSRGRGGPRCMSMPLVREDI

SEQ ID NO: 28 - protein, 408 aa, Mycoplasma sp.
MHVTSEIKKLKKVLVHRPGKELLNLTPDTLGRLLFDDIPYLKDAILEHDEFCQILRDNDVEVVYLEDLMAETLDENPQVKPSFIRQFIYEAGVRTPKYKDLLFDYLMSYTNNKELVLKTMEGIKVSEVHRNKQDSEYSLVDQISEETKFLAEPMPNLYFTRDPFASVGDGIILNKMHSVTRSRETIYAYYIFNYHPDYMDKVPKYYDRENPFSIEGGDVLNLNEHTLAIGISQRTSAEAIDLVAKNMFNDEKCNIDTILAFKIPECRAFMHLDTVFTQIDIDKFTYHPGIMDTLEVFEITKNEDDLDEVRVIKKEGSLENILEEYLGIDITLIPCAGGDKIASEREQWNDGTNTLCIAPGVVVVYNRNNITNEVLREKGIKVIEMNSAELSRGRGGPRCMSMPLERED